European Patent Specification EP 2 974 737 B1, published October 22, 2025. Title: TECHNIQUES FOR PREDICTING, DETECTING AND REDUCING ASPECIFIC PROTEIN INTERFERENCE IN ASSAYS INVOLVING IMMUNOGLOBULIN SINGLE VARIABLE DOMAINS. Applicant: Ablynx N.V. The sequence listing filed with the application follows.

SEQUENCE LISTING (89 sequences)

SEQ ID NO: 1 - protein, 270 aa, Artificial Sequence
  Nanobody, nanobody construct or other immunoglobulin single variable domain
EVQLVESGGGLVQPGGSLRLSCAASGFTFSSYAMSWVRQAPGKGLEWVSGIKSSGDSTRYAGSVKGRFTISRDNAKNTLYLQMNSLRPEDTAVYYCAKSRVSRTGLYTYDNRGQGTLVTVSSGGGGSGGGGSGGGGSGGGGSEVQLVESGGGLVQPGGSLRLSCAASGRTFNNYAMGWFRQAPGKEREFVAAITRSGVRSGVSAIYGDSVKDRFTISRDNAKNTLYLQMNSLRPEDTAVYYCAASAIGSGALRRFEYDYSGQGTLVTVSS

SEQ ID NO: 2 - protein, 385 aa, Artificial Sequence
  Nanobody, nanobody construct or other immunoglobulin single variable domain
EVQLVESGGGLVQPGGSLRLSCAASGFTFSSYPMGWFRQAPGKGREFVSSITGSGGSTYYADSVKGRFTISRDNAKNTLYLQMNSLRPEDTAVYYCAAYIRPDTYLSRDYRKYDYWGQGTLVTVSSGGGGSGGGSEVQLVESGGGLVQPGNSLRLSCAASGFTFSSFGMSWVRQAPGKGLEWVSSISGSGSDTLYADSVKGRFTISRDNAKTTLYLQMNSLRPEDTAVYYCTIGGSLSRSSQGTLVTVSSGGGGSGGGSEVQLVESGGGLVQPGGSLRLSCAASGFTFSSYPMGWFRQAPGKGREFVSSITGSGGSTYYADSVKGRFTISRDNAKNTLYLQMNSLRPEDTAVYYCAAYIRPDTYLSRDYRKYDYWGQGTLVTVSS

SEQ ID NO: 3 - protein, 117 aa, Artificial Sequence
  Nanobody, nanobody construct or other immunoglobulin single variable domain
EVQLVESGGGLVQAGGSLRLSCAASRSIGRLDRMGWYRHRTGEPRELVATITGGSSINYGDFVKGRFTISIDNAKNTVYLQMNNLKPEDTAVYYCNFNKYVTSRDTWGQGTQVTVSS

SEQ ID NO: 4 - protein, 140 aa, Artificial Sequence
  Nanobody, nanobody construct or other immunoglobulin single variable domain
EVQLVESGGGLVQAGGSLRLSCAASRSIGRLDRMGWYRHRTGEPRELVATITGGSSINYGDFVKGRFTISIDNAKNTVYLQMNNLKPEDTAVYYCNFNKYVTSRDTWGQGTQVTVSSAAAEQKLISEEDLNGAAHHHHHH

SEQ ID NO: 5 - protein, 117 aa, Artificial Sequence
  Nanobody, nanobody construct or other immunoglobulin single variable domain
EVQLVESGGGLVQPGGSLRLSCAASRSIGRLDRMGWYRHRPGEPRELVATITGGSSINYGDSVKGRFTISIDNSKNTVYLQMNSLRPEDTAVYYCNFNKYVTSRDTWGQGTLVTVSS

SEQ ID NO: 6 - protein, 125 aa, Artificial Sequence
  Nanobody, nanobody construct or other immunoglobulin single variable domain
HHHHHHEVQLVESGGGLVQPGGSLRLSCAASRSIGRLDRMGWYRHRPGEPRELVATITGGSSINYGDSVKGRFTISIDNSKNTVYLQMNSLRPEDTAVYYCNFNKYVTSRDTWGQGTLVTVSSAA

SEQ ID NO: 7 - protein, 124 aa, Artificial Sequence
  Nanobody, nanobody construct or other immunoglobulin single variable domain
HHHHHHEVQLVESGGGLVQPGGSLRLSCAASRSIGRLDRMGWYRHRPGEPRELVATITGGSSINYGDSVKGRFTISIDNSKNTVYLQMNSLRPEDTAVYYCNFNKYVTSRDTWGQGTLVTVSSA

SEQ ID NO: 8 - protein, 124 aa, Artificial Sequence
  Nanobody, nanobody construct or other immunoglobulin single variable domain
HHHHHHEVQLVESGGGLVQPGGSLRLSCAASRSIGRLDRMGWYRHRPGEPRELVATITGGSSINYGDSVKGRFTISIDNSKNTVYLQMNSLRPEDTAVYYCNFNKYVTSRDTWGQGTLVTVSSG

SEQ ID NO: 9 - protein, 125 aa, Artificial Sequence
  Nanobody, nanobody construct or other immunoglobulin single variable domain
HHHHHHEVQLVESGGGLVQPGGSLRLSCAASRSIGRLDRMGWYRHRPGEPRELVATITGGSSINYGDSVKGRFTISIDNSKNTVYLQMNSLRPEDTAVYYCNFNKYVTSRDTWGQGTLVTVSSGG

SEQ ID NO: 10 - protein, 126 aa, Artificial Sequence
  Nanobody, nanobody construct or other immunoglobulin single variable domain
HHHHHHEVQLVESGGGLVQPGGSLRLSCAASRSIGRLDRMGWYRHRPGEPRELVATITGGSSINYGDSVKGRFTISIDNSKNTVYLQMNSLRPEDTAVYYCNFNKYVTSRDTWGQGTLVTVSSGGG

SEQ ID NO: 11 - protein, 123 aa, Artificial Sequence
  Nanobody, nanobody construct or other immunoglobulin single variable domain
HHHHHHEVQLVESGGGLVQAGGSLRLSCAASRSIGRLDRMGWYRHRPGEPRELVATITGGSSINYGDSVKGRFTISIDNSKNTVYLQMNSLRPEDTAVYYCNFNKYVTSRDTWGQGTLVTVSS

SEQ ID NO: 12 - protein, 123 aa, Artificial Sequence
  Nanobody, nanobody construct or other immunoglobulin single variable domain
HHHHHHEVQLVESGGGLVQPGGSLRLSCAASRSIGRLDRMGWYRHRPGEPRELVATITGGSSINYGDSVKGRFTISIDNSKNTVYLQMNSLKPEDTAVYYCNFNKYVTSRDTWGQGTLVTVSS

SEQ ID NO: 13 - protein, 123 aa, Artificial Sequence
  Nanobody, nanobody construct or other immunoglobulin single variable domain
HHHHHHEVQLVESGGGLVQAGGSLRLSCAASRSIGRLDRMGWYRHRPGEPRELVATITGGSSINYGDSVKGRFTISIDNSKNTVYLQMNSLRPEDTAVYYCNFNKYVTSRDTWGQGTQVTVSS

SEQ ID NO: 14 - protein, 123 aa, Artificial Sequence
  Nanobody, nanobody construct or other immunoglobulin single variable domain
HHHHHHEVQLVESGGGLVQPGGSLRLSCAASRSIGRLDRMGWYRHRPGEPRELVATITGGSSINYGDSVKGRFTISIDNSKNTVYLQMNSLRPEDTAVYYCNFNKYVTSRDTWGQGTQVTVSS

SEQ ID NO: 15 - protein, 123 aa, Artificial Sequence
  Nanobody, nanobody construct or other immunoglobulin single variable domain
HHHHHHEVQLVESGGGLVQPGGSLRLSCAASRSIGRLDRMGWYRHRPGEPRELVATITGGSSINYGDSVKGRFTISIDNSKNTVYLQMNSLRPEDTAVYYCNFNKYVTSRDTWGQGTLVQVSS

SEQ ID NO: 16 - protein, 123 aa, Artificial Sequence
  Nanobody, nanobody construct or other immunoglobulin single variable domain
HHHHHHEVQLVESGGGSVQPGGSLRLSCAASRSIGRLDRMGWYRHRPGEPRELVATITGGSSINYGDSVKGRFTISIDNSKNTVYLQMNSLRPEDTAVYYCNFNKYVTSRDTWGQGTLVTVSS

SEQ ID NO: 17 - protein, 121 aa, Artificial Sequence [sequence omitted]

SEQ ID NO: 18 - protein, 146 aa, Artificial Sequence
  Nanobody, nanobody construct or other immunoglobulin single variable domain
EVQLVESGGGLVQPGGSLRLSCAASGSVFKINVMAWYRQAPGKGRELVAGIISGGSTSYADSVKGRFTISRDNAKNTLYLQMNSLRPEDTAVYYCAFITTESDYDLGRRYWGQGTLVTVSSGGGGSGGGSRDWDFDVFGGGTPVGG

SEQ ID NO: 19 - protein, 151 aa, Artificial Sequence
  Nanobody, nanobody construct or other immunoglobulin single variable domain
EVQLVESGGGLVQPGGSLRLSCIASGLPFSTKSMGWFRQAPGKEREFVARISPGGTSRYYGDFVKGRFAISRDNAKNTTWLQMNSLKAEDTAVYYCASGERSTYIGSNYYRTNEYDYWGTGTQVTVSSAAAEQKLISEEDLNGAAHHHHHH

SEQ ID NO: 20 - protein, 128 aa, Artificial Sequence
  Nanobody, nanobody construct or other immunoglobulin single variable domain
EVQLVESGGGLVQPGGSLRLSCIASGLPFSTKSMGWFRQAPGKEREFVARISPGGTSRYYGDFVKGRFAISRDNAKNTTWLQMNSLKAEDTAVYYCASGERSTYIGSNYYRTNEYDYWGTGTQVTVSS

SEQ ID NO: 21 - protein, 151 aa, Artificial Sequence
  Nanobody, nanobody construct or other immunoglobulin single variable domain
EVQLLESGGGLVQPGGSLRLSCAASGLPFSTKSMGWFRQAPGKGREFVSRISPGGTSRYYGDFVKGRFTISRDNSKNTLYLQMNSLRAEDTAVYYCASGERSTYIGSNYYRTNEYDYWGQGTLVTVSSAAAEQKLISEEDLNGAAHHHHHH

SEQ ID NO: 22 - protein, 128 aa, Artificial Sequence
  Nanobody, nanobody construct or other immunoglobulin single variable domain
EVQLLESGGGLVQPGGSLRLSCAASGLPFSTKSMGWFRQAPGKGREFVSRISPGGTSRYYGDFVKGRFTISRDNSKNTLYLQMNSLRAEDTAVYYCASGERSTYIGSNYYRTNEYDYWGQGTLVTVSS

SEQ ID NO: 23 - protein, 134 aa, Artificial Sequence
  Nanobody, nanobody construct or other immunoglobulin single variable domain
HHHHHHEVQLVESGGGLVQAGGSLRLSCAASGRTFNNYAMGWFRRAPGKEREFVAAITRSGVRSGVSAIYGDSVKDRFTISRDNAKNTLYLQMNSLKPEDTAVYTCAASAIGSGALRRFEYDYSGQGTQVTVSS

SEQ ID NO: 24 - protein, 134 aa, Artificial Sequence
  Nanobody, nanobody construct or other immunoglobulin single variable domain
HHHHHHEVQLVESGGGLVQPGGSLRLSCAASGRTFNNYAMGWFRRAPGKEREFVAAITRSGVRSGVSAIYGDSVKDRFTISRDNAKNTLYLQMNSLKPEDTAVYTCAASAIGSGALRRFEYDYSGQGTQVTVSS

SEQ ID NO: 25 - protein, 134 aa, Artificial Sequence
  Nanobody, nanobody construct or other immunoglobulin single variable domain
HHHHHHEVQLVESGGGLVQAGGSLRLSCAASGRTFNNYAMGWFRRAPGKEREFVAAITRSGVRSGVSAIYGDSVKDRFTISRDNAKNTLYLQMNSLRPEDTAVYTCAASAIGSGALRRFEYDYSGQGTQVTVSS

SEQ ID NO: 26 - protein, 134 aa, Artificial Sequence
  Nanobody, nanobody construct or other immunoglobulin single variable domain
HHHHHHEVQLVESGGGLVQAGGSLRLSCAASGRTFNNYAMGWFRRAPGKEREFVAAITRSGVRSGVSAIYGDSVKDRFTISRDNAKNTLYLQMNSLKPEDTAVYTCAASAIGSGALRRFEYDYSGQGTLVTVSS

SEQ ID NO: 27 - protein, 134 aa, Artificial Sequence
  Nanobody, nanobody construct or other immunoglobulin single variable domain
HHHHHHEVQLVESGGGLVQPGGSLRLSCAASGRTFNNYAMGWFRRAPGKEREFVAAITRSGVRSGVSAIYGDSVKDRFTISRDNAKNTLYLQMNSLRPEDTAVYTCAASAIGSGALRRFEYDYSGQGTLVTVSS

SEQ ID NO: 28 - protein, 134 aa, Artificial Sequence
  Nanobody, nanobody construct or other immunoglobulin single variable domain
HHHHHHEVQLVESGGGLVQPGGSLRLSCAASGRTFNNYAMGWFRQAPGKEREFVAAITRSGVRSGVSAIYGDSVKDRFTISRDNAKNTLYLQMNSLRPEDTAVYYCAASAIGSGALRRFEYDYSGQGTLVTVSS

SEQ ID NO: 29 - protein, 137 aa, Artificial Sequence
  Nanobody, nanobody construct or other immunoglobulin single variable domain
HHHHHHEVQLVESGGGLVQPGGSLRLSCAASGRTFNNYAMGWFRQAPGKEREFVAAITRSGVRSGVSAIYGDSVKDRFTISRDNAKNTLYLQMNSLRPEDTAVYYCAASAIGSGALRRFEYDYSGQGTLVTVSSAAA

SEQ ID NO: 30 - protein, 137 aa, Artificial Sequence; identical to SEQ ID NO: 29
  Nanobody, nanobody construct or other immunoglobulin single variable domain

SEQ ID NO: 31 - protein, 367 aa, Artificial Sequence
  Nanobody, nanobody construct or other immunoglobulin single variable domain
DVQLVESGGGLVQPGGSLRLSCAASRSIGRLDRMGWYRHRPGEPRELVATITGGSSINYGDSVKGRFTISIDNSKNTVYLQMNSLRPEDTAVYYCNFNKYVTSRDTWGQGTLVTVSSGGGGSGGGSEVQLVESGGGLVQPGNSLRLSCAASGFTFSSFGMSWVRQAPGKGLEWVSSISGSGSDTLYADSVKGRFTISRDNAKTTLYLQMNSLRPEDTAVYYCTIGGSLSRSSQGTLVTVSSGGGGSGGGSEVQLVESGGGLVQPGGSLRLSCAASRSIGRLDRMGWYRHRPGEPRELVATITGGSSINYGDSVKGRFTISIDNSKNTVYLQMNSLRPEDTAVYYCNFNKYVTSRDTWGQGTLVTVSS

SEQ ID NO: 32 - protein, 368 aa, Artificial Sequence
  Nanobody, nanobody construct or other immunoglobulin single variable domain
DVQLVESGGGLVQPGGSLRLSCAASRSIGRLDRMGWYRHRPGEPRELVATITGGSSINYGDSVKGRFTISIDNSKNTVYLQMNSLRPEDTAVYYCNFNKYVTSRDTWGQGTLVTVSSGGGGSGGGSEVQLVESGGGLVQPGNSLRLSCAASGFTFSSFGMSWVRQAPGKGLEWVSSISGSGSDTLYADSVKGRFTISRDNAKTTLYLQMNSLRPEDTAVYYCTIGGSLSRSSQGTLVTVSSGGGGSGGGSEVQLVESGGGLVQPGGSLRLSCAASRSIGRLDRMGWYRHRPGEPRELVATITGGSSINYGDSVKGRFTISIDNSKNTVYLQMNSLRPEDTAVYYCNFNKYVTSRDTWGQGTLVTVSSA

SEQ ID NO: 33 - protein, 5 aa, Artificial Sequence
  C-terminal sequence
VTVSS

SEQ ID NO: 34 - protein, 6 aa, Artificial Sequence
  C-terminal sequence
  MISC_FEATURE (6)..(6): X = a group (X)n, in which N = 1-10, preferably 1-5 and X is any amino acid.
VTVSSX

SEQ ID NO: 35 - protein, 218 aa, Artificial Sequence
  VH domain
QIQLVQSGPELKKPGETVKISCKASGYTFTAYSMHWVKQAPGKGLKWMGWINTVTGEPAYADDFKGRFAFSLETSASTAYLQISSLKNEDTATYFCTRGLIHFYYWGQGTTLTVSSAKTTPPSVYPLAPGSAAQTNSMVTLGCLVKGYFPEPVTVTWNSGSLSSGVHTFPAVLQSDLYTLSSSVTVPSSTWPSETVTCNVAHPASSTKVDKKIVPRDC

SEQ ID NO: 36 - protein, 214 aa, Artificial Sequence
  VK domain
DIQMTQTPSSLSASLGGRVTITCKASQDIHNFISWYQHKPGKVPRLIIHDTSTLQPGIPSRFSGSGSGRDYSFSITNLEPEDIATYYCLHYDNLLRSFGGGTKLEIKRADAAPTVSIFPPSSEQLTSGGASVVCFLNNFYPKDINVKWKIDGSERQNGVLNSWTDQDSKDSTYSMSSTLTLTKDEYERHNSYTCEATHKTSTSPIVKSFNRNEC

SEQ ID NO: 37 - protein, 122 aa, Artificial Sequence
  Nanobody, nanobody construct or other immunoglobulin single variable domain
HHHHHHEVQLVESGGGLVQPGNSLRLSCAASGFTFSSFGMSWVRQAPGKGLEWVSSISGSGSDTLYADSVKGRFTISRDNAKTTLYLQMNSLRPEDTAVYYCTIGGSLSRSSQGTLVTVSSA

SEQ ID NO: 38 - protein, 271 aa, Artificial Sequence
  Nanobody, nanobody construct or other immunoglobulin single variable domain
EVQLVESGGGLVQPGGSLRLSCAASGFTFSSYAMSWVRQAPGKGLEWVSGIKSSGDSTRYAGSVKGRFTISRDNAKNTLYLQMNSLRPEDTAVYYCAKSRVSRTGLYTYDNRGQGTLVTVSSGGGGSGGGGSGGGGSGGGGSEVQLVESGGGLVQPGGSLRLSCAASGRTFNNYAMGWFRQAPGKEREFVAAITRSGVRSGVSAIYGDSVKDRFTISRDNAKNTLYLQMNSLRPEDTAVYYCAASAIGSGALRRFEYDYSGQGTLVTVSSA

SEQ ID NO: 39 - protein, 386 aa, Artificial Sequence
  Nanobody or Nanobody construct
EVQLVESGGGLVQPGGSLRLSCAASGFTFSSYPMGWFRQAPGKGREFVSSITGSGGSTYYADSVKGRFTISRDNAKNTLYLQMNSLRPEDTAVYYCAAYIRPDTYLSRDYRKYDYWGQGTLVTVSSGGGGSGGGSEVQLVESGGGLVQPGNSLRLSCAASGFTFSSFGMSWVRQAPGKGLEWVSSISGSGSDTLYADSVKGRFTISRDNAKTTLYLQMNSLRPEDTAVYYCTIGGSLSRSSQGTLVTVSSGGGGSGGGSEVQLVESGGGLVQPGGSLRLSCAASGFTFSSYPMGWFRQAPGKGREFVSSITGSGGSTYYADSVKGRFTISRDNAKNTLYLQMNSLRPEDTAVYYCAAYIRPDTYLSRDYRKYDYWGQGTLVTVSSA

SEQ ID NO: 40 - protein, 364 aa, Artificial Sequence
  Nanobody, nanobody construct or other immunoglobulin single variable domain
EVQLVESGGGLVQPGGSLRLSCAASGFTFSDYWMYWVRQAPGKGLEWVSEINTNGLITKYPDSVKGRFTISRDNAKNTLYLQMNSLRPEDTAVYYCARSPSGFNRGQGTLVTVSSGGGGSGGGSEVQLVESGGGLVQPGNSLRLSCAASGFTFSSFGMSWVRQAPGKGLEWVSSISGSGSDTLYADSVKGRFTISRDNAKTTLYLQMNSLRPEDTAVYYCTIGGSLSRSSQGTLVTVSSGGGGSGGGSEVQLVESGGGLVQPGGSLRLSCAASGFTFSDYWMYWVRQAPGKGLEWVSEINTNGLITKYPDSVKGRFTISRDNAKNTLYLQMNSLRPEDTAVYYCARSPSGFNRGQGTLVTVSSA

SEQ ID NO: 41 - protein, 246 aa, Artificial Sequence
  Nanobody, nanobody construct or other immunoglobulin single variable domain
EVQLVESGGGLVQPGGSLRLSCAASGSVFKINVMAWYRQAPGKGRELVAGIISGGSTSYADSVKGRFTISRDNAKNTLYLQMNSLRPEDTAVYYCAFITTESDYDLGRRYWGQGTLVTVSSGGGGSGGGSEVQLVESGGGLVQPGNSLRLSCAASGFTFSSFGMSWVRQAPGKGLEWVSSISGSGSDTLYADSVKGRFTISRDNAKTTLYLQMNSLRPEDTAVYYCTIGGSLSRSSQGTLVTVSSA

SEQ ID NO: 42 - protein, 260 aa, Artificial Sequence
  Nanobody, nanobody construct or other immunoglobulin single variable domain
EVQLVESGGGLVQPGGSLRLSCAASGRTFSYNPMGWFRQAPGKGRELVAAISRTGGSTYYPDSVEGRFTISRDNAKRMVYLQMNSLRAEDTAVYYCAAAGVRAEDGRVRTLPSEYTFWGQGTQVTVSSAAAEVQLVESGGGLVQPGGSLRLSCAASGRTFSYNPMGWFRQAPGKGRELVAAISRTGGSTYYPDSVEGRFTISRDNAKRMVYLQMNSLRAEDTAVYYCAAAGVRAEDGRVRTLPSEYTFWGQGTQVTVSSA

SEQ ID NO: 43 - protein, 250 aa, Artificial Sequence
  Nanobody, nanobody construct or other immunoglobulin single variable domain
DVQLVESGGGLVQPGGSLRLSCAASGFILDYYAIGWFRQAPGKEREGVLCIDASDDITYYADSVKGRFTISRDNSKNTVYLQMNSLRPEDTAVYYCATPIGLSSSCLLEYDYDYWGQGTLVTVSSGGGGSGGGSEVQLLESGGGLVQPGGSLRLSCAASGFTFRSFGMSWVRQAPGKGPEWVSSISGSGSDTLYADSVKGRFTISRDNSKNTLYLQMNSLRPEDTAVYYCTIGGSLSRSSQGTLVTVSSA

SEQ ID NO: 44 - protein, 368 aa, Artificial Sequence; identical to SEQ ID NO: 32
  Nanobody, nanobody construct or other immunoglobulin single variable domain

SEQ ID NO: 45 - protein, 117 aa, Artificial Sequence; identical to SEQ ID NO: 3
  Nanobody, nanobody construct or other immunoglobulin single variable domain

SEQ ID NO: 46 - protein, 143 aa, Artificial Sequence
  Nanobody, nanobody construct or other immunoglobulin single variable domain
EVQLVESGGGLVQAGGSLRLSCAASRSIGRLDRMGWYRHRTGEPRELVATITGGSSINYGDFVKGRFTISIDNAKNTVYLQMNNLKPEDTAVYYCNFNKYVTSRDTWGQGTQVTVSSAAAHHHHHHGAAEQKLISEEDLNGAA

SEQ ID NO: 47 - protein, 146 aa, Artificial Sequence; identical to SEQ ID NO: 18
  Nanobody, nanobody construct or other immunoglobulin single variable domain

SEQ ID NO: 48 - protein, 151 aa, Artificial Sequence; identical to SEQ ID NO: 19
  Nanobody, nanobody construct or other immunoglobulin single variable domain

SEQ ID NO: 49 - protein, 151 aa, Artificial Sequence; identical to SEQ ID NO: 21
  Nanobody, nanobody construct or other immunoglobulin single variable domain

SEQ ID NO: 50 - protein, 121 aa, Artificial Sequence
  Nanobody, nanobody construct or other immunoglobulin single variable domain
HHHHHHEVQLVESGGGSVQPGNSLRLSCAASGFTFSSFGMSWVRQAPGKGLEWVSSISGSGSDTLYADSVKGRFTISRDNAKTTLYLQMNSLRPEDTAVYYCTIGGSLSRSSQGTLVTVSS

SEQ ID NO: 51 - protein, 121 aa, Artificial Sequence
  Nanobody, nanobody construct or other immunoglobulin single variable domain
HHHHHHEVQLVESGGGLVQPGNSLRLSCAASGFTFSSFGMSWVRQAPGKGLEWVSSISGSGSDTLYADSVKGRFTISRDNAKTTLYLQMNSLRPEDTAVYYCTIGGSLSRSSQGTLVQVSS

SEQ ID NO: 52 - protein, 121 aa, Artificial Sequence
  Nanobody, nanobody construct or other immunoglobulin single variable domain
HHHHHHEVQLVESGGGLVQPGNSLRLSCAASGFTFSSFGMSWVRQAPGKGLEWVSSISGSGSDTLYADSVKGRFTISRDNAKTTLYLQMNSLRPEDTAVYYCTIGGSLSRSSQGTLVTVGS

SEQ ID NO: 53 - protein, 121 aa, Artificial Sequence
  Nanobody, nanobody construct or other immunoglobulin single variable domain
HHHHHHEVQLVESGGGLVQPGNSLRLSCAASGFTFSSFGMSWVRQAPGKGLEWVSSISGSGSDTLYADSVKGRFTISRDNAKTTLYLQMNSLRPEDTAVYYCTIGGSLSRSSQGTLVTVSG

SEQ ID NO: 54 - protein, 121 aa, Artificial Sequence
  Nanobody, nanobody construct or other immunoglobulin single variable domain
HHHHHHEVQLVESGGGSVQPGNSLRLSCAASGFTFSSFGMSWVRQAPGKGLEWVSSISGSGSDTLYADSVKGRFTISRDNAKTTLYLQMNSLRPEDTAVYYCTIGGSLSRSSQGTLVQVGG

SEQ ID NO: 55 - protein, 122 aa, Artificial Sequence; identical to SEQ ID NO: 37
  Nanobody, nanobody construct or other immunoglobulin single variable domain

SEQ ID NO: 56 - protein, 123 aa, Artificial Sequence
  Nanobody, nanobody construct or other immunoglobulin single variable domain
HHHHHHEVQLVESGGGLVQPGNSLRLSCAASGFTFSSFGMSWVRQAPGKGLEWVSSISGSGSDTLYADSVKGRFTISRDNAKTTLYLQMNSLRPEDTAVYYCTIGGSLSRSSQGTLVTVSSGG

SEQ ID NO: 57 - protein, 123 aa, Artificial Sequence
  Nanobody, nanobody construct or other immunoglobulin single variable domain
HHHHHHEVQLVESGGGLVQPGNSLRLSCAASGFTFSSFGMSWVRQAPGKGLEWVSSISGSGSDTLYADSVKGRFTISRDNAKTTLYLQMNSLRPEDTAVYYCTIGGSLSRSSQGTLVTVSSAS

SEQ ID NO: 58 - protein, 124 aa, Artificial Sequence
  Nanobody, nanobody construct or other immunoglobulin single variable domain
HHHHHHEVQLVESGGGLVQPGNSLRLSCAASGFTFSSFGMSWVRQAPGKGLEWVSSISGSGSDTLYADSVKGRFTISRDNAKTTLYLQMNSLRPEDTAVYYCTIGGSLSRSSQGTLVTVSSAST

SEQ ID NO: 59 - protein, 125 aa, Artificial Sequence
  Nanobody, nanobody construct or other immunoglobulin single variable domain
HHHHHHEVQLVESGGGLVQPGNSLRLSCAASGFTFSSFGMSWVRQAPGKGLEWVSSISGSGSDTLYADSVKGRFTISRDNAKTTLYLQMNSLRPEDTAVYYCTIGGSLSRSSQGTLVTVSSASTK

SEQ ID NO: 60 - protein, 124 aa, Artificial Sequence
  Nanobody, nanobody construct or other immunoglobulin single variable domain
HHHHHHEVQLVESGGGLVQPGNSLRLSCAASGFTFSSFGMSWVRQAPGKGLEWVSSISGSGSDTLYADSVKGRFTISRDNAKTTLYLQMNSLRPEDTAVYYCTIGGSLSRSSQGTLVTVSSASP

SEQ ID NO: 61 - protein, 123 aa, Artificial Sequence
  Nanobody, nanobody construct or other immunoglobulin single variable domain
HHHHHHEVQLVESGGGLVQPGNSLRLSCAASGFTFSSFGMSWVRQAPGKGLEWVSSISGSGSDTLYADSVKGRFTISRDNAKTTLYLQMNSLRPEDTAVYYCTIGGSLSRSSQGTLVTVSSAP

SEQ ID NO: 62 - protein, 124 aa, Artificial Sequence
  Nanobody, nanobody construct or other immunoglobulin single variable domain
HHHHHHEVQLVESGGGLVQPGNSLRLSCAASGFTFSSFGMSWVRQAPGKGLEWVSSISGSGSDTLYADSVKGRFTISRDNAKTTLYLQMNSLRPEDTAVYYCTIGGSLSRSSQGTLVTVSSAPT

SEQ ID NO: 63 - protein, 122 aa, Artificial Sequence
  Nanobody, nanobody construct or other immunoglobulin single variable domain
HHHHHHEVQLVESGGGLVQPGNSLRLSCAASGFTFSSFGMSWVRQAPGKGLEWVSSISGSGSDTLYADSVKGRFTISRDNAKTTLYLQMNSLRPEDTAVYYCTIGGSLSRSSQGTLVTVSSW

SEQ ID NO: 64 - protein, 122 aa, Artificial Sequence
  Nanobody, nanobody construct or other immunoglobulin single variable domain
HHHHHHEVQLVESGGGLVQPGNSLRLSCAASGFTFSSFGMSWVRQAPGKGLEWVSSISGSGSDTLYADSVKGRFTISRDNAKTTLYLQMNSLRPEDTAVYYCTIGGSLSRSSQGTLVTVSSL

SEQ ID NO: 65 - protein, 123 aa, Artificial Sequence; identical to SEQ ID NO: 11
  Nanobody, nanobody construct or other immunoglobulin single variable domain

SEQ ID NO: 66 - protein, 123 aa, Artificial Sequence; identical to SEQ ID NO: 16
  Nanobody, nanobody construct or other immunoglobulin single variable domain

SEQ ID NO: 67 - protein, 123 aa, Artificial Sequence; identical to SEQ ID NO: 12
  Nanobody, nanobody construct or other immunoglobulin single variable domain

SEQ ID NO: 68 - protein, 123 aa, Artificial Sequence; identical to SEQ ID NO: 13
  Nanobody, nanobody construct or other immunoglobulin single variable domain

SEQ ID NO: 69 - protein, 123 aa, Artificial Sequence; identical to SEQ ID NO: 14
  Nanobody, nanobody construct or other immunoglobulin single variable domain

SEQ ID NO: 70 - protein, 123 aa, Artificial Sequence; identical to SEQ ID NO: 15
  Nanobody, nanobody construct or other immunoglobulin single variable domain

SEQ ID NO: 71 - protein, 123 aa, Artificial Sequence
  Nanobody, nanobody construct or other immunoglobulin single variable domain
HHHHHHEVQLVESGGGLVQPGGSLRLSCAASRSIGRLDRMGWYRHRPGEPRELVATITGGSSINYGDSVKGRFTISIDNSKNTVYLQMNSLRPEDTAVYYCNFNKYVTSRDTWGQGTLVTVSG

SEQ ID NO: 72 - protein, 123 aa, Artificial Sequence
  Nanobody, nanobody construct or other immunoglobulin single variable domain
HHHHHHEVQLVESGGGLVQPGGSLRLSCAASRSIGRLDRMGWYRHRPGEPRELVATITGGSSINYGDSVKGRFTISIDNSKNTVYLQMNSLRPEDTAVYYCNFNKYVTSRDTWGQGTLVTVGG

SEQ ID NO: 73 - protein, 124 aa, Artificial Sequence
  Nanobody, nanobody construct or other immunoglobulin single variable domain
HHHHHHEVQLVESGGGLVQPGGSLRLSCAASRSIGRLDRMGWYRHRPGEPRELVATITGGSSINYGDSVKGRFTISIDNSKNTVYLQMNSLRPEDTAVYYCNFNKYVTSRDTWGQGTLVTVGGG

SEQ ID NO: 74 - protein, 124 aa, Artificial Sequence; identical to SEQ ID NO: 8
  Nanobody, nanobody construct or other immunoglobulin single variable domain

SEQ ID NO: 75 - protein, 125 aa, Artificial Sequence; identical to SEQ ID NO: 6
  Nanobody, nanobody construct or other immunoglobulin single variable domain

SEQ ID NO: 76 - protein, 126 aa, Artificial Sequence; identical to SEQ ID NO: 10
  Nanobody, nanobody construct or other immunoglobulin single variable domain

SEQ ID NO: 77 - protein, 124 aa, Artificial Sequence; identical to SEQ ID NO: 7
  Nanobody, nanobody construct or other immunoglobulin single variable domain

SEQ ID NO: 78 - protein, 123 aa, Artificial Sequence
  Nanobody, nanobody construct or other immunoglobulin single variable domain
HHHHHHEVQLVESGGGLVRPGGSLRLSCAASRSIGRLDRMGWYRHRPGEPRELVATITGGSSINYGDSVKGRFTISIDNSKNTVYLQMNSLRPEDTAVYYCNFNKYVTSRDTWGQGTLVTVSS

SEQ ID NO: 79 - protein, 124 aa, Artificial Sequence
  Nanobody, nanobody construct or other immunoglobulin single variable domain
HHHHHEVQLVESGGGLVQPGGSLRLSCAASRSIGRLDRMGWYRHRPGEPRELVATITGGSSINYGDSVKGRFTISIDNSKNTVYLQMNSLRPEDTAVYYCNFNKYVTSRDTWGQGTLVTVSSGG

SEQ ID NO: 80 - protein, 123 aa, Artificial Sequence
  Nanobody, nanobody construct or other immunoglobulin single variable domain
HHHHHHEVQLVESGGGLVQPGGSLRLSCAASRSIGRLDRMGWYRHRPGEPRELVATITGGSSINYGDSVKGRFTISIDNSKNTVYLQMNSLRPEDTAVYYCNFNKYVTSRDTWGQGTLVQVGG

SEQ ID NO: 81 - protein, 123 aa, Artificial Sequence
  Nanobody, nanobody construct or other immunoglobulin single variable domain
HHHHHHEVQLVESGGGVVQPGGSLRLSCAASRSIGRLDRMGWYRHRPGEPRELVATITGGSSINYGDSVKGRFTISIDNSKNTVYLQMNSLRPEDTAVYYCNFNKYVTSRDTWGQGTLVTVSS

SEQ ID NO: 82 - protein, 123 aa, Artificial Sequence
  Nanobody, nanobody construct or other immunoglobulin single variable domain
HHHHHHEVQLVESGGGLVQPGGSLRLSCAASRSIGRLDRMGWYRHRPGEPRELVATITGGSSINYGDSVKGRFTISIDNSKNTVYLQMNSLRAEDTAVYYCNFNKYVTSRDTWGQGTLVTVSS

SEQ ID NO: 83 - protein, 123 aa, Artificial Sequence
  Nanobody, nanobody construct or other immunoglobulin single variable domain
HHHHHHEVQLVESGGGLVQPGGSLRLSCAASRSIGRLDRMGWYRHRPGEPRELVATITGGSSINYGDSVKGRFTISIDNSKNTVYLQMNSLRPEDAAVYYCNFNKYVTSRDTWGQGTLVTVSS

SEQ ID NO: 84 - protein, 123 aa, Artificial Sequence
  Nanobody, nanobody construct or other immunoglobulin single variable domain
HHHHHHEVQLVESGGGLVQPGGSLRLSCAASRSIGRLDRMGWYRHRPGEPRELVATITGGSSINYGDSVKGRFTISIDNSKNTVYLQMNSLRPEDTAVYYCNFNKYVTSRDTWGQGTLVTVGS

SEQ ID NO: 85 - protein, 123 aa, Artificial Sequence
  Nanobody, nanobody construct or other immunoglobulin single variable domain
HHHHHHEVQLVESGGGSVQPGGSLRLSCAASRSIGRLDRMGWYRHRPGEPRELVATITGGSSINYGDSVKGRFTISIDNSKNTVYLQMNSLRPEDTAVYYCNFNKYVTSRDTWGQGTLVQVGG

SEQ ID NO: 86 - protein, 123 aa, Artificial Sequence
  Nanobody, nanobody construct or other immunoglobulin single variable domain
HHHHHHEVQLVESGGGSVQPGGSLRLSCAASRSIGRLDRMGWYRHRPGEPRELVATITGGSSINYGDSVKGRFTISIDNSKNTVYLQMNSLRPEDTAVYYCNFNKYVTSRDTWGQGTLVQVSS

SEQ ID NO: 87 - protein, 123 aa, Artificial Sequence
  Nanobody, nanobody construct or other immunoglobulin single variable domain
HHHHHHEVQLVESGGGSVQPGGSLRLSCAASRSIGRLDRMGWYRHRPGEPRELVATITGGSSINYGDSVKGRFTISIDNSKNTVYLQMNSLRPEDTAVYYCNFNKYVTSRDTWGQGTLVTVGG

SEQ ID NO: 88 - protein, 124 aa, Artificial Sequence
  Nanobody, nanobody construct or other immunoglobulin single variable domain
HHHHHHEVQLVESGGGSVQPGGSLRLSCAASRSIGRLDRMGWYRHRPGEPRELVATITGGSSINYGDSVKGRFTISIDNSKNTVYLQMNSLRPEDTAVYYCNFNKYVTSRDTWGQGTLVQVSSA

SEQ ID NO: 89 - protein, 123 aa, Artificial Sequence
  Nanobody, nanobody construct or other immunoglobulin single variable domain
HHHHHHEVQLVESGGGSVQAGGSLRLSCAASRSIGRLDRMGWYRHRPGEPRELVATITGGSSINYGDSVKGRFTISIDNSKNTVYLQMNSLRPEDTAVYYCNFNKYVTSRDTWGQGTLVQVGG